European Patent Application EP 4 219 506 A1, published August 2, 2023. Title: PROTECTED DYE-LABELED REAGENTS. Applicant: Pacific Biosciences of California, Inc. Application EP. The sequence listing filed with the application follows.

SEQUENCE LISTING (26 sequences)

SEQ ID NO: 1 - protein, 575 aa, Bacteriophage phi-29 [sequence omitted]

SEQ ID NO: 2 - protein, 572 aa, Bacteriophage M2Y
MSRKMFSCDFETTTKLDDCRVWAYGYMEIGNLDNYKIGNSLDEFMQWVMEIQADLYFHNLKFDGAFIVNWLEQHGFKWSNEGLPNTYNTIISKMGQWYMIDICFGYKGKRKLHTVIYDSLKKLPFPVKKIAKDFQLPLLKGDIDYHTERPVGHEITPEEYEYIKNDIEIIARALDIQFKQGLDRMTAGSDSLKGFKDILSTKKFNKVFPKLSLPMDKEIRKAYRGGFTWLNDKYKEKEIGEGMVFDVNSLYPSQMYSRPLPYGAPIVFQGKYEKDEQYPLYIQRIRFEFELKEGYIPTIQIKKNPFFKGNEYLKNSGVEPVELYLTNVDLELIQEHYELYNVEYIDGFKFREKTGLFKDFIDKWTYVKTHEEGAKKQLAKLMLNSLYGKFASNPDVTGKVPYLKDDGSLGFRVGDEEYKDPVYTPMGVFITAWARFTTITAAQACYDRIIYCDTDSIHLTGTEVPEIIKDIVDPKKLGYWAHESTFKRAKYLRQKTYIQDIYVKEVDGKLKECSPDEATTTKFSVKCAGMTDTIKKKVTFDNFAVGFSSMGKPKPVQVNGGVVLVDSVFTIK

SEQ ID NO: 3 - protein, 572 aa, Bacteriophage B103
MPRKMFSCDFETTTKLDDCRVWAYGYMEIGNLDNYKIGNSLDEFMQWVMEIQADLYFHNLKFDGAFIVNWLEHHGFKWSNEGLPNTYNTIISKMGQWYMIDICFGYKGKRKLHTVIYDSLKKLPFPVKKIAKDFQLPLLKGDIDYHAERPVGHEITPEEYEYIKNDIEIIARALDIQFKQGLDRMTAGSDSLKGFKDILSTKKFNKVFPKLSLPMDKEIRRAYRGGFTWLNDKYKEKEIGEGMVFDVNSLYPSQMYSRPLPYGAPIVFQGKYEKDEQYPLYIQRIRFEFELKEGYIPTIQIKKNPFFKGNEYLKNSGAEPVELYLTNVDLELIQEHYEMYNVEYIDGFKFREKTGLFKEFIDKWTYVKTHEKGAKKQLAKLMFDSLYGKFASNPDVTGKVPYLKEDGSLGFRVGDEEYKDPVYTPMGVFITAWARFTTITAAQACYDRIIYCDTDSIHLTGTEVPEIIKDIVDPKKLGYWAHESTFKRAKYLRQKTYIQDIYAKEVDGKLIECSPDEATTTKFSVKCAGMTDTIKKKVTFDNFRVGFSSTGKPKPVQVNGGVVLVDSVFTIK

SEQ ID NO: 4 - protein, 578 aa, Bacteriophage GA-1
MARSVYVCDFETTTDPEDCRLWAWGWMDIYNTDKWSYGEDIDSFMEWALNSNSDIYFHNLKFDGSFILPWWLRNGYVHTEEDRTNTPKEFTTTISGMGQWYAVDVCINTRGKNKNHVVFYDSLKKLPFKVEQIAKGFGLPVLKGDIDYKKYRPVGYVMDDNEIEYLKHDLLIVALALRSMFDNDFTSMTVGSDALNTYKEMLGVKQWEKYFPVLSLKVNSEIRKAYKGGFTWVNPKYQGETVYGGMVFDVNSMYPAMMKNKLLPYGEPVMFKGEYKKNVEYPLYIQQVRCFFELKKDKIPCIQIKGNARFGQNEYLSTSGDEYVDLYVTNVDWELIKKHYDIFEEEFIGGFMFKGFIGFFDEYIDRFMEIKNSPDSSAEQSLQAKLMLNSLYGKFATNPDITGKVPYLDENGVLKFRKGELKERDPVYTPMGCFITAYARENILSNAQKLYPRFIYADTDSIHVEGLGEVDAIKDVIDPKKLGYWDHEATFQRARYVRQKTYFIETTWKENDKGKLVVCEPQDATKVKPKIACAGMSDAIKERIRFNEFKIGYSTHGSLKPKNVLGGVVLMDYPFAIK

SEQ ID NO: 5 - protein, 566 aa, Bacteriophage AV-1
MVRQSTIASPARGGVRRSHKKVPSFCADFETTTDEDDCRVWSWGIIQVGKLQNYVDGISLDGFMSHISERASHIYFHNLAFDGTFILDWLLKHGYRWTKENPGVKEFTSLISRMGKYYSITVVFETGFRVEFRDSFKKLPMSVSAIAKAFNLHDQKLEIDYEKPRPIGYIPTEQEKRYQRNDVAIVAQALEVQFAEKMTKLTAGSDSLATYKKMTGKLFIRRFPILSPEIDTEIRKAYRGGFTYADPRYAKKLNGKGSVYDVNSLYPSVMRTALLPYGEPIYSEGAPRTNRPLYIASITFTAKLKPNHIPCIQIKKNLSFNPTQYLEEVKEPTTVVATNIDIELWKKHYDFKIYSWNGTFEFRGSHGFFDTYVDHFMEIKKNSTGGLRQIAKLHLNSLYGKFATNPDITGKHPTLKDNRVSLVMNEPETRDPVYTPMGVFITAYARKKTISAAQDNYETFAYADTDSLHLIGPTTPPDSLWVDPVELGAWKHESSFTKSVYIRAKQYAEEIGGKLDVHIAGMPRNVAATLTLEDMLHGGTWNGKLIPVRVPGGTVLKDTTFTLKID

SEQ ID NO: 6 - protein, 568 aa, Bacteriophage CP-1
MTCYYAGDFETTTNEEETEVWLSCFAKVIDYDKLDTFKVNTSLEDFLKSLYLDLDKTYTETGEDEFIIFFHNLKFDGSFLLSFFLNNDIECTYFINDMGVWYSITLEFPDFTLTFRDSLKILNFSIATMAGLFKMPIAKGTTPLLKHKPEVIKPEWIDYIHVDVAILARGIFAMYYEENFTKYTSASEALTEFKRIFRKSKRKFRDFFPILDEKVDDFCRKHIVGAGRLPTLKHRGRTLNQLIDIYDINSMYPATMLQNALPIGIPKRYKGKPKEIKEDHYYIYHIKADFDLKRGYLPTIQIKKKLDALRIGVRTSDYVTTSKNEVIDLYLTNFDLDLFLKHYDATIMYVETLEFQTESDLFDDYITTYRYKKENAQSPAEKQKAKIMLNSLYGKFGAKIISVKKLAYLDDKGILRFKNDDEEEVQPVYAPVALFVTSIARHFIISNAQENYDNFLYADTDSLHLFHSDSLVLDIDPSEFGKWAHEGRAVKAKYLRSKLYIEELIQEDGTTHLDVKGAGMTPEIKEKITFENFVIGATFEGKRASKQIKGGTLIYETTFKIRETDYLV

SEQ ID NO: 7 - protein, 650 aa, synthetic construct
  REGION 1..650: note = Mutant recombinant phi29-type DNA polymerase
MKHMPRKMYSCDFETTTKVEDCRVWAYGYMNIEDHSEYKIGNSLDEFMAWVLKVQADLYFHNLKFDGSFIINWLERNGFKWSADGLPNTYNTIISRMGQWYMIDISLGYKGKRKIHTVIYDSLKKLPFPVKKIAQDFKLTVRKGDIDYHKERPVGYKITPEEYAYIKNDIQIIAEALLIQFKQGLDRMTAGSDSLKGFKDIITTKKFKKVFPTLSLGLDKEVRKAYRGGFTWLNDRFKGKEIGEGMVFDINSAYPAQMYSRLLPYGEPIVFEGKYVWDEDYPLHIQHIRCEFELKEGYIPTIQIKQSLFYKGNEYLKSSGGEIADLWLSNVDLELMKEHYDLYNVEYISGLKFKATTGLFKDFIDKWSYIKTTSWGAIKQLAKLMLNSLYGKFASNPDVTGKVPYLKENGALGFRLGEEEYKDPVYTPMGVFITAWGRYTTITAAQACYDRIIYCDTDSIHLTGTKIPDVIKDIVHPKKLGYWEHESTFKRAKYLRQKTYIQDIYMKRVRGFLVQGSPDDYTDIKFSVKCAGMTDKIKEEVTFENFKVGFSRKMKPKAVQVPGGVVLVDSVFTIKGGGSLVPRGSGGGSGGGSGGGSGLNDFFEAQKIEWHEGGGSGGGSGGGSGLNDFFEAQKIEWHEGHHHHHHHHHH

SEQ ID NO: 8 - protein, 640 aa, synthetic construct
  REGION 1..640: note = Mutant recombinant phi29-type DNA polymerase
MKHMPRKMYSCDFETTTKVEDCRVWAYGYMNIEDHSEYKIGNSLDEFMAWVLKVQADLYFHNLKFDGSFIINWLERNGFKWSADGLPNTYNTIISRMGQWYMIDICLGYKGKRKIHTVIYDSLKKLPFPVKKIARDFKLTVKKGDIDYHKERPVGYKITPEEYAYIKNDIQIIAEALLIQFKQGLDRMTAGSDSLKGFKDIITTKKFKKVFPTLSLGLDKEVRKAYRGGFTWLNDRFKGKEIGEGMVFDINSAYPAQMYSKLLPYGEPIVFEGKYVWDEDYPLHIQHIRCEFELKEGYIPTIQIKQSLFYKGNEYLKSSGGEIADVWLSNVDLELMKEHYDLYNVEYISGLKFKATTGLFKDFIDKWSYIKTTSWGAIKQLAKLMLNSLYGKFASNPDVTGKVPYLKENGALGFRLGEEEYKDPVYTPMGVFITAYGRWTIITAAQAVYDRIIYCDTDSIHLTGTKIPDVIKDIVHPKKLGYWEHESTFKRAKYLRQKTYIQDIYMKQVRGHLVQGSPDDYTDIKFSVKCAGMTDKIKEEVTFENFKVGFSRKMKPKAVQVPGGVVLVDSVFTIKGHHHHHHHHHHGGGSGGGSGGGSGLNDFFEAQKIEWHEGGGSGGGSGGGSGLNDFFEAQKIEWHE

SEQ ID NO: 9 - protein, 650 aa, synthetic construct
  REGION 1..650: note = Mutant recombinant phi29-type DNA polymerase
MKHMPRKMYSCDFETTTKVEDCRVWAYGYMNIEDHSEYKIGNSLDEFMAWVLKVQADLYFHNLKFDGSFIINWLERNGFKWSADGLPNTYNTIISRMGQWYMIDISLGYKGKRKIHTVIYDSLKKLPFPVKKISRDFKLTVKKGDIDYHKERPVGYKITPEEYAYIKNDIQIIAEALLIQFKQGLDRMTAGSDSLKGFKDIITTKKFKKVFPTLSLGLDKEVRKAYRGGFTWLNDRFKGKEIGEGMVFDINSAYPAQMYSKLLPYGEPIVFEGKYVWDEDYPLHIQHIRCEFELKEGYIPTIQIKQSLFYKGNEYLKSSGGEIADVWLSNVDLELMKEHYDLYNVEYISGLKFKATTGLFKDFIDKWTYIKTTSFGAIKQLAKLMLNSLYGKFASNPDVTGKVPYLKENGALGFRLGEEEYKDPVYTPMGVFITAYGRWTTITAAQACYDRIIYCDTDSIHLTGTKIPDVIKDIVHPKKLGYWEHESTFKRAKYLRQKTYIQDIYMKRVRGFLVQGSPDDYTDIKFSVKCAGMTDKIKEEVTFENFKVGFSRKMKPKAVQVPGGVVLVDSVFTIKGGGSLVPRGSGGGSGGGSGGGSGLNDFFEAQKIEWHEGGGSGGGSGGGSGLNDFFEAQKIEWHEGHHHHHHHHHH

SEQ ID NO: 10 - protein, 640 aa, synthetic construct
  REGION 1..640: note = Mutant recombinant phi29-type DNA polymerase
MKHMPRKMYSCDFETTTKVEDCRVWAYGYMNIEDHSEYKIGNSLDEFMAWVLKVQADLYFHNLKFDGSFIINWLERNGFKWSADGLPNTYNTIISRMGQWYMIDICLGYKGKRKIHTVIYDSLKKLPFPVKKIAKDFKLTVKKGDIDYHKERPVGYKITPEEYAYIKNDIQIIAEALLIQFKQGLDRMTAGSDSLKGFKDIITTKKFKKVFPTLSLGLDKEVRKAYRGGFTWLNDRFKGKEIGEGMVFDINSAYPAQMYSRLLPYGEPIVFEGKYVWDEDYPLHIQHIRCEFELKEGYIPTIQIKQSLFYKGNEYLKSSGGEIADLWLSNVDLELMKEHYDLYNVEYISGLKFKATTGLFKDFIDKWSYIKTTSWGAIKQLAKLMLNSLYGKFASNPDVTGKVPYLKENGALGFRLGEEEYKDPVYTPMGVFITAWGRYTTITAAQACYDRIIYCDTDSIHLTGTKIPDVIKDIVHPKKLGYWEHESTFKRAKYLRQKTYIQDIYMKRVKGFLVQGSPDDYTDIKFSVKCAGMTDKIKEEVTFENFKVGFSRKMKPKAVQVPGGVVLVDSVFTIKGGGSGGGSGGGSGLNDFFEAQKIEWHEGGGSGGGSGGGSGLNDFFEAQKIEWHEGHHHHHHHHHH

SEQ ID NO: 11 - protein, 640 aa, synthetic construct
  REGION 1..640: note = Mutant recombinant phi29-type DNA polymerase
MKHMPRKMYSCDFETTTKVEDCRVWAYGYMNIEDHSEYKIGNSLDEFMAWVLKVQADLYFHNLKFDGSFIINWLERNGFKWSADGLPNTYNTIISRMGQWYMIDISLGYKGKRKIHTVIYDSLKKLPFPVKKIAQDFKLTVKKGDIDYHKERPVGYKITPEEYAYIKNDIQIIAEALLIQFKQGLDRMTAGSDSLKGFKDIITTKKFKKVFPTLSLGLDKEVRKAYRGGFTWLNDRFKGKEIGEGMVFDINSAYPAQMYSKLLPYGEPIVFEGKYVWDEDYPLHIQHIRCEFELKEGYIPTIQIKQSLFYKGNEYLKSSGGEIADVWLSNVDLELMKEHYDLYNVEYISGLKFKATTGLFKDFIDKWTYIKTTSWGAIKQLAKLMLNSLYGKFASNPDVTGKVPYLKENGALGFRLGEEEYKDPVYTPMGVFITAYGRWTTITAAQACYDRIIYCDTDSIHLTGTKIPDVIKDIVHPKKLGYWEHESTFKRAKYLRQKTYIQDIYMKRVRGYLVQGSPDDYTDIKFSVKCAGMTDKIKEEVTFENFKVGFSRKMKPKAVQVPGGVVLVDSVFTIKGGGSGGGSGGGSGLNDFFEAQKIEWHEGGGSGGGSGGGSGLNDFFEAQKIEWHEGHHHHHHHHHH

SEQ ID NO: 12 - protein, 640 aa, synthetic construct
  REGION 1..640: note = Mutant recombinant phi29-type DNA polymerase
MKHMPRKMYSCDFETTTKVEDCRVWAYGYMNIEDHSEYKIGNSLDEFMAWVLKVQADLYFHNLKFDGSFIINWLERNGFKWSADGLPNTYNTIISRMGQWYMIDICLGYKGKRKIHTVIYDSLKKLPFPVKKIARDFKLTVKKGDIDYHKERPVGYKITPEEYAYIKNDIQIIAEALLIQFKQGLDRMTAGSDSLKGFKDIITTKKFKKVFPTLSLGLDKEVRKAYRGGFTWLNDRFKGKEIGEGMVFDINSAYPAQMYSKLLPYGEPIVFEGKYVWDEDYPLHIQHIRCEFELKEGYIPTIQIKQSLFYKGNEYLKSSGGEIADVWLSNVDLELMKEHYDLYNVEYISGLKFKATTGLFKDFIDKWTYIKTTSWGAIKQLAKLMLNSLYGKFASNPDVTGKVPYLKENGALGFRLGEEEYKDPVYTPMGVFITAYGRWTTITAAQACYDRIIYCDTDSIHLTGTKIPDVIKDIVDPKKLGYWEHESTFKRAKYLRQKTYIQDIYMKRVRGHLVQGSPDDYTDIKFSVKCAGMTDKIKEEVTFENFKVGFSRKMKPKAVQVPGGVVLVDSVFTIKGHHHHHHHHHHGGGSGGGSGGGSGLNDFFEAQKIEWHEGGGSGGGSGGGSGLNDFFEAQKIEWHE

SEQ ID NO: 13 - protein, 650 aa, synthetic construct
  REGION 1..650: note = Mutant recombinant phi29-type DNA polymerase
MKHMPRKMYSCDFETTTKVEDCRVWAYGYMNIEDHSEYKIGNSLDEFMAWVLKVQADLYFHNLKFDGSFIINWLERNGFKWSADGLPNTYNTIISRMGQWYMIDISLGYKGKRKIHTVIYDSLKKLPFPVKKIAQDFKLTVKKGDIDYHKERPVGYKITPEEYAYIKNDIQIIAEALLIQFKQGLDRMTAGSDSLKGFKDIITTKKFKKVFPTLSLGLDKEVRKAYRGGFTWLNDRFKGKEIGEGMVFDINSAYPAQMYSKLLPYGEPIVFEGKYVWDEDYPLHIQHIRCEFELKEGYIPTIQIKQSLFYKGNEYLKSSGGEIADVWLSNVDLELMKEHYDLYNVEYISGLKFKATTGLFKDFIDKWTYIKTFSYGAIKQLAKLMLNSLYGKFASNPDVTGKVPYLKENGALGFRLGEEEYKDPVYTPMGVFITAYGRWTTITAAQACYDRIIYCDTDSIHLTGTKIPDVIKDIVHPKKLGYWEHESTFKRAKYLRQKTYIQDIYMKRVRGYLVQGSPDDYTDIKFSVKCAGMTDKIKEEVTFENFKVGFSRKMKPKAVQVPGGVVLVDSVFTIKGGGSLVPRGSGGGSGGGSGGGSGLNDFFEAQKIEWHEGGGSGGGSGGGSGLNDFFEAQKIEWHEGHHHHHHHHHH

SEQ ID NO: 14 - protein, 640 aa, synthetic construct
  REGION 1..640: note = Mutant recombinant phi29-type DNA polymerase
MKHMPRKMYSCDFETTTKVEDCRVWAYGYMNIEDHSEYKIGNSLDEFMAWVLKVQADLYFHNLKFDGSFIINWLERNGFKWSADGLPNTYNTIISRMGQWYMIDICLGYKGKRKIHTVIYDSLKKLPFPVKKIAQDFKLTVKKGDIDYHKERPVGYKITPEEYAYIKNDIQIIAEALLIQFKQGLDRMTAGSDSLKGFKDIITTKKFKKVFPTLSLGLDKEVRKAYRGGFTWLNDRFKGKEIGEGMVFDINSAYPAQMYSKLLPYGEPIVFEGKYVWDEDYPLHIQHIRCEFELKEGYIPTIQIKQSLFYKGNEYLKSSGGEIADVWLSNVDLELMKEHYDLYNVEYISGLKFKATTGLFKDFIDKWTYIKTTSYGAIKQLAKLMLNSLYGKFASNPDVTGKVPYLKENGALGFRLGEEEYKDPVYTPMGVFITAYGRWTTITAAQACYDRIIYCDTDSIHLTGTKIPDVIKDIVHPKKLGYWEHESTFKRAKYLRQKTYIQDIYMKRVRGYLVQGSPDDYTDIKFSVKCAGMTDKIKEEVTFENFKVGFSRKMKPKAVQVPGGVVLVDSVFTIKGHHHHHHHHHHGGGSGGGSGGGSGLNDFFEAQKIEWHEGGGSGGGSGGGSGLNDFFEAQKIEWHE

SEQ ID NO: 15 - protein, 640 aa, synthetic construct
  REGION 1..640: note = Mutant recombinant phi29-type DNA polymerase
MKHMPRKMYSCDFETTTKVEDCRVWAYGYMNIEDHSEYKIGNSLDEFMAWVLKVQADLYFHNLKFDGSFIINWLERNGFKWSADGLPNTYNTIISRMGQWYMIDICLGYKGKRKIHTVIYDSLKKLPFPVKKIAQDFKLTVKKGDIDYHKERPVGYKITPEEYAYIKNDIQIIAEALLIQFKQGLDRMTAGSDSLKGFKDIITTKKFKKVFPTLSLGLDKEVRKAYRGGFTWLNDRFKGKEIGEGMVFDINSAYPAQMYSRLLPYGEPIVFEGKYVWDEDYPLHIQHIRCEFELKEGYIPTIQIKQSLFYKGNEYLKSSGGEIADLWLSNVDLELMKEHYDLYNVEYISGLKFKATTGLFKDFIDKWSYIKTTSYGAIKQLAKLMLNSLYGKFASNPDVTGKVPYLKENGALGFRLGEEEYKDPVYTPMGVFITAWGRYTTITAAQACYDRIIYCDTDSIHLTGTKIPDVIKDIVHPKKLGYWEHESTFKRAKYLRQKTYIQDIYMKRVRGYLVQGSPDDYTDIKFSVKCAGMTDKIKEEVTFENFKVGFSRKMKPKAVQVPGGVVLVDSVFTIKGGGSGGGSGGGSGLNDFFEAQKIEWHEGGGSGGGSGGGSGLNDFFEAQKIEWHEGHHHHHHHHHH

SEQ ID NO: 16 - protein, 640 aa, synthetic construct
  REGION 1..640: note = Mutant recombinant phi29-type DNA polymerase
MKHMPRKMYSCDFETTTKVEDCRVWAYGYMNIEDHSEYKIGNSLDEFMAWVLKVQADLYFHNLKFDGSFIINWLERNGFKWSADGLPNTYNTIISRMGQWYMIDICLGYKGKRKIHTVIYDSLKKLPFPVKKIAQDFKLTVKKGDIDYHKERPVGYKITPEEYAYIKNDIQIIAEALLIQFKQGLDRMTAGSDSLKGFKDIITTKKFKKVFPTLSLGLDKEVRKAYRGGFTWLNDRFKGKEIGEGMVFDINSAYPAQMYSRLLPYGEPIVFEGKYVWDEDYPLHIQHIRCEFELKEGYIPTIQIKQSLFYKGNEYLKSSGGEIADLWLSNVDLELMKEHYDLYNVEYISGLKFKATTGLFKDFIDKWSYIKTTSYGAIKQLAKLMLNSLYGKFASNPDVTGKVPYLKENGALGFRLGEEEYKDPVYTPMGVFITAWGRYTTITAAQACYDRIIYCDTDSIHLTGTKIPDVIKDIVHPKKLGYWEHESTFKRAKYLRQKTYIQDIYMKRVRGYLVQGSPDDYTDIKFSVKCAGMTDKIKEEVTFENFKVGFSRKMKPKAVQVPGGVVLVDSVFTIKGHHHHHHHHHHGGGSGGGSGGGSGLNDFFEAQKIEWHEGGGSGGGSGGGSGLNDFFEAQKIEWHE

SEQ ID NO: 17 - protein, 575 aa, synthetic construct
  REGION 1..575: note = Mutant recombinant phi29-type DNA polymerase
MKHMPRKMYSCDFETTTKVEDCRVWAYGYMNIEDHSEYKIGNSLDEFMAWVLKVQADLYFHNLKFDGSFIINWLERNGFKWSADGLPNTYNTIISRMGQWYMIDISLGYKGKRKIHTVIYDSLKKLPFPVKKIAQDFKLTVRKGDIDYHKERPVGYKITPEEYAYIKNDIQIIAEALLIQFKQGLDRMTAGSDSLKGFKDIITTKKFKKVFPTLSLGLDKEVRKAYRGGFTWLNDRFKGKEIGEGMVFDINSAYPAQMYSRLLPYGEPIVFEGKYVWDEDYPLHIQHIRCEFELKEGYIPTIQIKQSLFYKGNEYLKSSGGEIADLWLSNVDLELMKEHYDLYNVEYISGLKFKATTGLFKDFIDKWSYIKTTSWGAIKQLAKLMLNSLYGKFASNPDVTGKVPYLKENGALGFRLGEEEYKDPVYTPMGVFITAWGRYTTITAAQACYDRIIYCDTDSIHLTGTKIPDVIKDIVHPKKLGYWEHESTFKRAKYLRQKTYIQDIYMKRVRGFLVQGSPDDYTDIKFSVKCAGMTDKIKEEVTFENFKVGFSRKMKPKAVQVPGGVVLVDSVFTIK

SEQ ID NO: 18 - protein, 575 aa, synthetic construct
  REGION 1..575: note = Mutant recombinant phi29-type DNA polymerase
MKHMPRKMYSCDFETTTKVEDCRVWAYGYMNIEDHSEYKIGNSLDEFMAWVLKVQADLYFHNLKFDGSFIINWLERNGFKWSADGLPNTYNTIISRMGQWYMIDICLGYKGKRKIHTVIYDSLKKLPFPVKKIARDFKLTVKKGDIDYHKERPVGYKITPEEYAYIKNDIQIIAEALLIQFKQGLDRMTAGSDSLKGFKDIITTKKFKKVFPTLSLGLDKEVRKAYRGGFTWLNDRFKGKEIGEGMVFDINSAYPAQMYSKLLPYGEPIVFEGKYVWDEDYPLHIQHIRCEFELKEGYIPTIQIKQSLFYKGNEYLKSSGGEIADVWLSNVDLELMKEHYDLYNVEYISGLKFKATTGLFKDFIDKWSYIKTTSWGAIKQLAKLMLNSLYGKFASNPDVTGKVPYLKENGALGFRLGEEEYKDPVYTPMGVFITAYGRWTIITAAQAVYDRIIYCDTDSIHLTGTKIPDVIKDIVHPKKLGYWEHESTFKRAKYLRQKTYIQDIYMKQVRGHLVQGSPDDYTDIKFSVKCAGMTDKIKEEVTFENFKVGFSRKMKPKAVQVPGGVVLVDSVFTIK

SEQ ID NO: 19 - protein, 575 aa, synthetic construct
  REGION 1..575: note = Mutant recombinant phi29-type DNA polymerase
MKHMPRKMYSCDFETTTKVEDCRVWAYGYMNIEDHSEYKIGNSLDEFMAWVLKVQADLYFHNLKFDGSFIINWLERNGFKWSADGLPNTYNTIISRMGQWYMIDISLGYKGKRKIHTVIYDSLKKLPFPVKKISRDFKLTVKKGDIDYHKERPVGYKITPEEYAYIKNDIQIIAEALLIQFKQGLDRMTAGSDSLKGFKDIITTKKFKKVFPTLSLGLDKEVRKAYRGGFTWLNDRFKGKEIGEGMVFDINSAYPAQMYSKLLPYGEPIVFEGKYVWDEDYPLHIQHIRCEFELKEGYIPTIQIKQSLFYKGNEYLKSSGGEIADVWLSNVDLELMKEHYDLYNVEYISGLKFKATTGLFKDFIDKWTYIKTTSFGAIKQLAKLMLNSLYGKFASNPDVTGKVPYLKENGALGFRLGEEEYKDPVYTPMGVFITAYGRWTTITAAQACYDRIIYCDTDSIHLTGTKIPDVIKDIVHPKKLGYWEHESTFKRAKYLRQKTYIQDIYMKRVRGFLVQGSPDDYTDIKFSVKCAGMTDKIKEEVTFENFKVGFSRKMKPKAVQVPGGVVLVDSVFTIK

SEQ ID NO: 20 - protein, 575 aa, synthetic construct
  REGION 1..575: note = Mutant recombinant phi29-type DNA polymerase
MKHMPRKMYSCDFETTTKVEDCRVWAYGYMNIEDHSEYKIGNSLDEFMAWVLKVQADLYFHNLKFDGSFIINWLERNGFKWSADGLPNTYNTIISRMGQWYMIDICLGYKGKRKIHTVIYDSLKKLPFPVKKIAKDFKLTVKKGDIDYHKERPVGYKITPEEYAYIKNDIQIIAEALLIQFKQGLDRMTAGSDSLKGFKDIITTKKFKKVFPTLSLGLDKEVRKAYRGGFTWLNDRFKGKEIGEGMVFDINSAYPAQMYSRLLPYGEPIVFEGKYVWDEDYPLHIQHIRCEFELKEGYIPTIQIKQSLFYKGNEYLKSSGGEIADLWLSNVDLELMKEHYDLYNVEYISGLKFKATTGLFKDFIDKWSYIKTTSWGAIKQLAKLMLNSLYGKFASNPDVTGKVPYLKENGALGFRLGEEEYKDPVYTPMGVFITAWGRYTTITAAQACYDRIIYCDTDSIHLTGTKIPDVIKDIVHPKKLGYWEHESTFKRAKYLRQKTYIQDIYMKRVKGFLVQGSPDDYTDIKFSVKCAGMTDKIKEEVTFENFKVGFSRKMKPKAVQVPGGVVLVDSVFTIK

SEQ ID NO: 21 - protein, 575 aa, synthetic construct
  REGION 1..575: note = Mutant recombinant phi29-type DNA polymerase
MKHMPRKMYSCDFETTTKVEDCRVWAYGYMNIEDHSEYKIGNSLDEFMAWVLKVQADLYFHNLKFDGSFIINWLERNGFKWSADGLPNTYNTIISRMGQWYMIDISLGYKGKRKIHTVIYDSLKKLPFPVKKIAQDFKLTVKKGDIDYHKERPVGYKITPEEYAYIKNDIQIIAEALLIQFKQGLDRMTAGSDSLKGFKDIITTKKFKKVFPTLSLGLDKEVRKAYRGGFTWLNDRFKGKEIGEGMVFDINSAYPAQMYSKLLPYGEPIVFEGKYVWDEDYPLHIQHIRCEFELKEGYIPTIQIKQSLFYKGNEYLKSSGGEIADVWLSNVDLELMKEHYDLYNVEYISGLKFKATTGLFKDFIDKWTYIKTTSWGAIKQLAKLMLNSLYGKFASNPDVTGKVPYLKENGALGFRLGEEEYKDPVYTPMGVFITAYGRWTTITAAQACYDRIIYCDTDSIHLTGTKIPDVIKDIVHPKKLGYWEHESTFKRAKYLRQKTYIQDIYMKRVRGYLVQGSPDDYTDIKFSVKCAGMTDKIKEEVTFENFKVGFSRKMKPKAVQVPGGVVLVDSVFTIK

SEQ ID NO: 22 - protein, 575 aa, synthetic construct
  REGION 1..575: note = Mutant recombinant phi29-type DNA polymerase
MKHMPRKMYSCDFETTTKVEDCRVWAYGYMNIEDHSEYKIGNSLDEFMAWVLKVQADLYFHNLKFDGSFIINWLERNGFKWSADGLPNTYNTIISRMGQWYMIDICLGYKGKRKIHTVIYDSLKKLPFPVKKIARDFKLTVKKGDIDYHKERPVGYKITPEEYAYIKNDIQIIAEALLIQFKQGLDRMTAGSDSLKGFKDIITTKKFKKVFPTLSLGLDKEVRKAYRGGFTWLNDRFKGKEIGEGMVFDINSAYPAQMYSKLLPYGEPIVFEGKYVWDEDYPLHIQHIRCEFELKEGYIPTIQIKQSLFYKGNEYLKSSGGEIADVWLSNVDLELMKEHYDLYNVEYISGLKFKATTGLFKDFIDKWTYIKTTSWGAIKQLAKLMLNSLYGKFASNPDVTGKVPYLKENGALGFRLGEEEYKDPVYTPMGVFITAYGRWTTITAAQACYDRIIYCDTDSIHLTGTKIPDVIKDIVDPKKLGYWEHESTFKRAKYLRQKTYIQDIYMKRVRGHLVQGSPDDYTDIKFSVKCAGMTDKIKEEVTFENFKVGFSRKMKPKAVQVPGGVVLVDSVFTIK

SEQ ID NO: 23 - protein, 575 aa, synthetic construct
  REGION 1..575: note = Mutant recombinant phi29-type DNA polymerase
MKHMPRKMYSCDFETTTKVEDCRVWAYGYMNIEDHSEYKIGNSLDEFMAWVLKVQADLYFHNLKFDGSFIINWLERNGFKWSADGLPNTYNTIISRMGQWYMIDISLGYKGKRKIHTVIYDSLKKLPFPVKKIAQDFKLTVKKGDIDYHKERPVGYKITPEEYAYIKNDIQIIAEALLIQFKQGLDRMTAGSDSLKGFKDIITTKKFKKVFPTLSLGLDKEVRKAYRGGFTWLNDRFKGKEIGEGMVFDINSAYPAQMYSKLLPYGEPIVFEGKYVWDEDYPLHIQHIRCEFELKEGYIPTIQIKQSLFYKGNEYLKSSGGEIADVWLSNVDLELMKEHYDLYNVEYISGLKFKATTGLFKDFIDKWTYIKTFSYGAIKQLAKLMLNSLYGKFASNPDVTGKVPYLKENGALGFRLGEEEYKDPVYTPMGVFITAYGRWTTITAAQACYDRIIYCDTDSIHLTGTKIPDVIKDIVHPKKLGYWEHESTFKRAKYLRQKTYIQDIYMKRVRGYLVQGSPDDYTDIKFSVKCAGMTDKIKEEVTFENFKVGFSRKMKPKAVQVPGGVVLVDSVFTIK

SEQ ID NO: 24 - protein, 575 aa, synthetic construct
  REGION 1..575: note = Mutant recombinant phi29-type DNA polymerase
MKHMPRKMYSCDFETTTKVEDCRVWAYGYMNIEDHSEYKIGNSLDEFMAWVLKVQADLYFHNLKFDGSFIINWLERNGFKWSADGLPNTYNTIISRMGQWYMIDICLGYKGKRKIHTVIYDSLKKLPFPVKKIAQDFKLTVKKGDIDYHKERPVGYKITPEEYAYIKNDIQIIAEALLIQFKQGLDRMTAGSDSLKGFKDIITTKKFKKVFPTLSLGLDKEVRKAYRGGFTWLNDRFKGKEIGEGMVFDINSAYPAQMYSKLLPYGEPIVFEGKYVWDEDYPLHIQHIRCEFELKEGYIPTIQIKQSLFYKGNEYLKSSGGEIADVWLSNVDLELMKEHYDLYNVEYISGLKFKATTGLFKDFIDKWTYIKTTSYGAIKQLAKLMLNSLYGKFASNPDVTGKVPYLKENGALGFRLGEEEYKDPVYTPMGVFITAYGRWTTITAAQACYDRIIYCDTDSIHLTGTKIPDVIKDIVHPKKLGYWEHESTFKRAKYLRQKTYIQDIYMKRVRGYLVQGSPDDYTDIKFSVKCAGMTDKIKEEVTFENFKVGFSRKMKPKAVQVPGGVVLVDSVFTIK

SEQ ID NO: 25 - protein, 575 aa, synthetic construct
  REGION 1..575: note = Mutant recombinant phi29-type DNA polymerase
MKHMPRKMYSCDFETTTKVEDCRVWAYGYMNIEDHSEYKIGNSLDEFMAWVLKVQADLYFHNLKFDGSFIINWLERNGFKWSADGLPNTYNTIISRMGQWYMIDICLGYKGKRKIHTVIYDSLKKLPFPVKKIAQDFKLTVKKGDIDYHKERPVGYKITPEEYAYIKNDIQIIAEALLIQFKQGLDRMTAGSDSLKGFKDIITTKKFKKVFPTLSLGLDKEVRKAYRGGFTWLNDRFKGKEIGEGMVFDINSAYPAQMYSRLLPYGEPIVFEGKYVWDEDYPLHIQHIRCEFELKEGYIPTIQIKQSLFYKGNEYLKSSGGEIADLWLSNVDLELMKEHYDLYNVEYISGLKFKATTGLFKDFIDKWSYIKTTSYGAIKQLAKLMLNSLYGKFASNPDVTGKVPYLKENGALGFRLGEEEYKDPVYTPMGVFITAWGRYTTITAAQACYDRIIYCDTDSIHLTGTKIPDVIKDIVHPKKLGYWEHESTFKRAKYLRQKTYIQDIYMKRVRGYLVQGSPDDYTDIKFSVKCAGMTDKIKEEVTFENFKVGFSRKMKPKAVQVPGGVVLVDSVFTIK

SEQ ID NO: 26 - protein, 575 aa, synthetic construct; identical to SEQ ID NO: 25
  REGION 1..575: note = Mutant recombinant phi29-type DNA polymerase